European Patent Specification EP 3 785 724 B1, published September 2, 2026. Title: Glucagon and GLP-1 co-agonist compounds. Applicant: Eli Lilly and Company. The sequence listing filed with the application follows.

SEQUENCE LISTING (11 sequences)

SEQ ID NO: 1 - protein, 37 aa, Homo sapien
HSQGTFTSDYSKYLDSRRAQDFVQWLMNTKRNRNNIA

SEQ ID NO: 2 - protein, 34 aa, Artificial Sequence
  Synthetic Construct
  MISC_FEATURE (2)..(2): Xaa at position 2 is nonnaturally occurring amino acid 2-Aminoisobutyric Acid
  MOD_RES (2)..(2): Aib
  MOD_RES (20)..(20): Lys at position 20 is chemically modified by conjugation of the epsilon-amino group of the Lys side chain with a C14-C24 fatty acid via (i) a direct bond or (ii) a linker between the Lys at position 20 and the C14-C24 fatty acid
  MISC_FEATURE (28)..(28): Xaa at position 28 is Glu or Ser
  MOD_RES (34)..(34): Gly at position 34 is optionally amidated
HXQGTFTSDYSKYLDEKKAKEFVEWLLXGGPSSG

SEQ ID NO: 3 - protein, 34 aa, Artificial Sequence
  Synthetic Construct
  MISC_FEATURE (2)..(2): Xaa at position 2 is nonnaturally occurring amino acid 2-Aminoisobutyric Acid
  MOD_RES (2)..(2): Aib
  MOD_RES (20)..(20): Lys at position 20 is chemically modified by conjugation of the epsilon-amino group of the Lys side chain with a C14-C24 fatty acid via (i) a direct bond or (ii) a linker between the Lys at position 20 and the C14-C24 fatty acid
  MOD_RES (34)..(34): Gly at position 34 is optionally amidated
HXQGTFTSDYSKYLDEKKAKEFVEWLLEGGPSSG

SEQ ID NO: 4 - protein, 34 aa, Artificial Sequence
  Synthetic Construct
  MISC_FEATURE (2)..(2): Xaa at position 2 is nonnaturally occurring amino acid 2-Aminoisobutyric Acid
  MOD_RES (2)..(2): Aib
  MOD_RES (20)..(20): Lys at position 20 is chemically modified by conjugation of the epsilon-amino group of the Lys side chain with a C14-C24 fatty acid via (i) a direct bond or (ii) a linker between the Lys at position 20 and the C14-C24 fatty acid
  MOD_RES (34)..(34): Gly at position 34 is optionally amidated
HXQGTFTSDYSKYLDEKKAKEFVEWLLSGGPSSG

SEQ ID NO: 5 - protein, 34 aa, Artificial Sequence; identical to SEQ ID NO: 3
  Synthetic Construct
  MISC_FEATURE (2)..(2): Xaa at position 2 is nonnaturally occurring amino acid 2-Aminoisobutyric Acid
  MOD_RES (2)..(2): Aib
  MOD_RES (20)..(20): Lys at position 20 is chemically modified by conjugation of the epsilon-amino group of the Lys side chain with ([2-(2-aminoethoxy)-ethoxy]-acetyl)2-(y-Glu)-CO-(CH2)16CO2H
  MOD_RES (34)..(34): Gly at position 34 is amidated

SEQ ID NO: 6 - protein, 34 aa, Artificial Sequence; identical to SEQ ID NO: 3
  Synthetic Construct
  MISC_FEATURE (2)..(2): Xaa at position 2 is a nonnaturally occurring amino acid 2-Aminoisobutyric Acid
  MOD_RES (2)..(2): Aib
  MOD_RES (20)..(20): Lys at position 20 is chemically modified by conjugation of the epsilon-amino group of the Lys side chain with ([2-(2-aminoethoxy)-ethoxy]-acetyl)2-(y-Glu)-CO-(CH2)18CO2H
  MOD_RES (34)..(34): Gly at position 34 is amidated

SEQ ID NO: 7 - protein, 34 aa, Artificial Sequence; identical to SEQ ID NO: 4
  Synthetic Construct
  MISC_FEATURE (2)..(2): Xaa at position 2 is nonnaturally occurring amino acid 2-Aminoisobutyric Acid
  MOD_RES (2)..(2): Aib
  MOD_RES (20)..(20): Lys at position 20 is chemically modified by conjugation of the epsilon-amino group of the Lys side chain with ([2-(2-aminoethoxy)-ethoxy]-acetyl)2-(y-Glu)2-CO-(CH2)16CO2H
  MOD_RES (34)..(34): Gly at position 34 is amidated

SEQ ID NO: 8 - protein, 34 aa, Artificial Sequence; identical to SEQ ID NO: 4
  Synthetic Construct
  MISC_FEATURE (2)..(2): Xaa at position 2 is nonnaturally occurring amino acid 2-aminoisobutyric Acid
  MOD_RES (2)..(2): Aib
  MOD_RES (20)..(20): Lys at position 20 is chemically modified by conjugation of the epsilon-amino group of the Lys side chain with ([2-(2-aminoethoxy)-ethoxy]-acetyl)2-(y-Glu)2-CO-(CH2)18CO2H
  MOD_RES (34)..(34): Gly at position 34 is amidated

SEQ ID NO: 9 - protein, 34 aa, Artificial Sequence; identical to SEQ ID NO: 2
  Synthetic Construct
  MISC_FEATURE (2)..(2): Xaa at position 2 is nonnaturally occurring amino acid 2-aminoisobutyric Acid
  MOD_RES (2)..(2): Aib
  MISC_FEATURE (28)..(28): Xaa at position 28 is Glu or Ser
  MOD_RES (34)..(34): Gly at position 34 is optionally amidated

SEQ ID NO: 10 - protein, 34 aa, Artificial Sequence; identical to SEQ ID NO: 3
  Synthetic Construct
  MISC_FEATURE (2)..(2): Xaa at position 2 is nonnaturally occurring amino acid 2-aminoisobutyric Acid
  MOD_RES (2)..(2): Aib
  MOD_RES (34)..(34): Gly at position 34 is optionally amidated

SEQ ID NO: 11 - protein, 34 aa, Artificial Sequence; identical to SEQ ID NO: 4
  Synthetic Construct
  MISC_FEATURE (2)..(2): Xaa at position 2 is nonnaturally occurring amino acid 2-aminoisobutyric Acid
  MOD_RES (2)..(2): Aib
  MOD_RES (34)..(34): Gly at position 34 is optionally amidated